European Patent Specification EP 3 695 906 B1, published August 2, 2023. Title: Probentransferwerkzeug. Applicant: Axagarius GmbH & Co. KG. The sequence listing filed with the application follows.

SEQUENCE LISTING (32 sequences)

SEQ ID NO: 1 - DNA, 20 bp, primer
ggaatggcattgacttggtc

SEQ ID NO: 2 - DNA, 19 bp, primer
gttctcggaaccgatcaca

SEQ ID NO: 3 - DNA, 20 bp, primer
ctgaagcttttggctttgag

SEQ ID NO: 4 - DNA, 19 bp, primer
ccgctgccaaattctttgg

SEQ ID NO: 5 - DNA, 18 bp, primer
aacgaccccttcattgac

SEQ ID NO: 6 - DNA, 19 bp, primer
tccacgacatactcagcac

SEQ ID NO: 7 - DNA, 15 bp, primer
ctcctacctctacaa

SEQ ID NO: 8 - DNA, 16 bp, primer
ggctagtgttaggaat

SEQ ID NO: 9 - DNA, 22 bp, primer
gagatgtttttgctggtattga

SEQ ID NO: 10 - DNA, 23 bp, primer
aaygtataaaccaatgcttccat

SEQ ID NO: 11 - DNA, 19 bp, primer
gacgggaattgaacccgcg

SEQ ID NO: 12 - DNA, 22 bp, primer
gttatgcatgaacgtaatgctc

SEQ ID NO: 13 - DNA, 22 bp, primer
gccctctactccacccccatcc

SEQ ID NO: 14 - DNA, 23 bp, primer
gcccatctgcaagcctttttgtg

SEQ ID NO: 15 - DNA, 25 bp, primer
ccgctgtatcacaagggctggtacc

SEQ ID NO: 16 - DNA, 25 bp, primer
ggagcccgtgtagagcatgacgatc

SEQ ID NO: 17 - DNA, 23 bp, primer
gtaacttccaaattcagagaaac

SEQ ID NO: 18 - DNA, 24 bp, primer
tctctaatttagaattagaaggaa

SEQ ID NO: 19 - DNA, 21 bp, primer
cacagtatttgctcgctgaga

SEQ ID NO: 20 - DNA, 19 bp, primer
ccattgctgcttcttctcc

SEQ ID NO: 21 - DNA, 24 bp, primer
ttaattcaaaaatcatttttcccg

SEQ ID NO: 22 - DNA, 22 bp, primer
tcaatgaaagtcccattctttg

SEQ ID NO: 23 - DNA, 18 bp, primer
ttccgaaccgaatcaagg

SEQ ID NO: 24 - DNA, 17 bp, primer
ggagcaccgttccaagc

SEQ ID NO: 25 - DNA, 19 bp, primer
cawcgatgaagaacgyagc

SEQ ID NO: 26 - DNA, 20 bp, primer
rgtttcttttcctccgctta

SEQ ID NO: 27 - DNA, 22 bp, primer
ggaagkaraagtcgtaacaagg

SEQ ID NO: 28 - DNA, 20 bp, primer
rgtttcttttcctccgctta

SEQ ID NO: 29 - DNA, 22 bp, primer
ccttatcayttagaggaaggag

SEQ ID NO: 30 - DNA, 20 bp, primer
rgtttcttttcctccgctta

SEQ ID NO: 31 - DNA, 28 bp, primer
ctagaggagcctgttctataatcgataa

SEQ ID NO: 32 - DNA, 25 bp, primer
tgacctaacgtctttatgtgtggtg